European Patent Application EP 4 148 144 A1, published March 15, 2023. Title: Composition for distinguishing of erythropoietin gene doping and use thereof. Applicant: KOREA INSTITUTE OF SCIENCE AND TECHNOLOGY. The sequence listing filed with the application follows.

SEQUENCE LISTING (9 sequences)

SEQ ID NO: 1 - RNA, 117 nt, Artificial Sequence
  sgRNA 1
uaauacgacucacuauagggacattcgtgcacccccaguuuuagagcuagaaauagcaaguuaaaauaaggcuaguccguuaucaacuugaaaaaguggcaccgagucggugcuuuu

SEQ ID NO: 2 - RNA, 118 nt, Artificial Sequence
  sgRNA 2
uaauacgacucacuauaggaggccgagaatatcacgacguuuuagagcuagaaauagcaaguuaaaauaaggcuaguccguuaucaacuugaaaaaguggcaccgagucggugcuuuu

SEQ ID NO: 3 - RNA, 118 nt, Artificial Sequence
  sgRNA 3
uaauacgacucacuauagcctggaagaggatggaggtcguuuuagagcuagaaauagcaaguuaaaauaaggcuaguccguuaucaacuugaaaaaguggcaccgagucggugcuuuu

SEQ ID NO: 4 - RNA, 118 nt, Artificial Sequence
  sgRNA 4
uaauacgacucacuauagtcgggctctgggagcccagaguuuuagagcuagaaauagcaaguuaaaauaaggcuaguccguuaucaacuugaaaaaguggcaccgagucggugcuuuu

SEQ ID NO: 5 - protein, 1403 aa, Artificial Sequence
  dCas9-3XFLAG
MGSSHHHHHHSSGDKKYSIGLAIGTNSVGWAVITDEYKVPSKKFKVLGNTDRHSIKKNLIGALLFDSGETAEATRLKRTARRRYTRRKNRICYLQEIFSNEMAKVDDSFFHRLEESFLVEEDKKHERHPIFGNIVDEVAYHEKYPTIYHLRKKLVDSTDKADLRLIYLALAHMIKFRGHFLIEGDLNPDNSDVDKLFIQLVQTYNQLFEENPINASGVDAKAILSARLSKSRRLENLIAQLPGEKKNGLFGNLIALSLGLTPNFKSNFDLAEDAKLQLSKDTYDDDLDNLLAQIGDQYADLFLAAKNLSDAILLSDILRVNTEITKAPLSASMIKRYDEHHQDLTLLKALVRQQLPEKYKEIFFDQSKNGYAGYIDGGASQEEFYKFIKPILEKMDGTEELLVKLNREDLLRKQRTFDNGSIPHQIHLGELHAILRRQEDFYPFLKDNREKIEKILTFRIPYYVGPLARGNSRFAWMTRKSEETITPWNFEEVVDKGASAQSFIERMTNFDKNLPNEKVLPKHSLLYEYFTVYNELTKVKYVTEGMRKPAFLSGEQKKAIVDLLFKTNRKVTVKQLKEDYFKKIECFDSVEISGVEDRFNASLGTYHDLLKIIKDKDFLDNEENEDILEDIVLTLTLFEDREMIEERLKTYAHLFDDKVMKQLKRRRYTGWGRLSRKLINGIRDKQSGKTILDFLKSDGFANRNFMQLIHDDSLTFKEDIQKAQVSGQGDSLHEHIANLAGSPAIKKGILQTVKVVDELVKVMGRHKPENIVIEMARENQTTQKGQKNSRERMKRIEEGIKELGSQILKEHPVENTQLQNEKLYLYYLQNGRDMYVDQELDINRLSDYDVDAIVPQSFLKDDSIDNKVLTRSDKNRGKSDNVPSEEVVKKMKNYWRQLLNAKLITQRKFDNLTKAERGGLSELDKAGFIKRQLVETRQITKHVAQILDSRMNTKYDENDKLIREVKVITLKSKLVSDFRKDFQFYKVREINNYHHAHDAYLNAVVGTALIKKYPKLESEFVYGDYKVYDVRKMIAKSEQEIGKATAKYFFYSNIMNFFKTEITLANGEIRKRPLIETNGETGEIVWDKGRDFATVRKVLSMPQVNIVKKTEVQTGGFSKESILPKRNSDKLIARKKDWDPKKYGGFDSPTVAYSVLVVAKVEKGKSKKLKSVKELLGITIMERSSFEKNPIDFLEAKGYKEVKKDLIIKLPKYSLFELENGRKRMLASAGELQKGNELALPSKYVNFLYLASHYEKLKGSPEDNEQKQLFVEQHKHYLDEIIEQISEFSKRVILADANLDKVLSAYNKHRDKPIREQAENIIHLFTLTNLGAPAAFKYFDTTIDRKRYTSTKEVLDATLIHQSITGLYETRIDLSQLGGDGDYKDHDGDYKDHDIDYKDDDDK

SEQ ID NO: 6 - protein, 1380 aa, Artificial Sequence
  dCas9 for dCas9-biotin
MGSSHHHHHHSSGDKKYSIGLAIGTNSVGWAVITDEYKVPSKKFKVLGNTDRHSIKKNLIGALLFDSGETAEATRLKRTARRRYTRRKNRICYLQEIFSNEMAKVDDSFFHRLEESFLVEEDKKHERHPIFGNIVDEVAYHEKYPTIYHLRKKLVDSTDKADLRLIYLALAHMIKFRGHFLIEGDLNPDNSDVDKLFIQLVQTYNQLFEENPINASGVDAKAILSARLSKSRRLENLIAQLPGEKKNGLFGNLIALSLGLTPNFKSNFDLAEDAKLQLSKDTYDDDLDNLLAQIGDQYADLFLAAKNLSDAILLSDILRVNTEITKAPLSASMIKRYDEHHQDLTLLKALVRQQLPEKYKEIFFDQSKNGYAGYIDGGASQEEFYKFIKPILEKMDGTEELLVKLNREDLLRKQRTFDNGSIPHQIHLGELHAILRRQEDFYPFLKDNREKIEKILTFRIPYYVGPLARGNSRFAWMTRKSEETITPWNFEEVVDKGASAQSFIERMTNFDKNLPNEKVLPKHSLLYEYFTVYNELTKVKYVTEGMRKPAFLSGEQKKAIVDLLFKTNRKVTVKQLKEDYFKKIECFDSVEISGVEDRFNASLGTYHDLLKIIKDKDFLDNEENEDILEDIVLTLTLFEDREMIEERLKTYAHLFDDKVMKQLKRRRYTGWGRLSRKLINGIRDKQSGKTILDFLKSDGFANRNFMQLIHDDSLTFKEDIQKAQVSGQGDSLHEHIANLAGSPAIKKGILQTVKVVDELVKVMGRHKPENIVIEMARENQTTQKGQKNSRERMKRIEEGIKELGSQILKEHPVENTQLQNEKLYLYYLQNGRDMYVDQELDINRLSDYDVDAIVPQSFLKDDSIDNKVLTRSDKNRGKSDNVPSEEVVKKMKNYWRQLLNAKLITQRKFDNLTKAERGGLSELDKAGFIKRQLVETRQITKHVAQILDSRMNTKYDENDKLIREVKVITLKSKLVSDFRKDFQFYKVREINNYHHAHDAYLNAVVGTALIKKYPKLESEFVYGDYKVYDVRKMIAKSEQEIGKATAKYFFYSNIMNFFKTEITLANGEIRKRPLIETNGETGEIVWDKGRDFATVRKVLSMPQVNIVKKTEVQTGGFSKESILPKRNSDKLIARKKDWDPKKYGGFDSPTVAYSVLVVAKVEKGKSKKLKSVKELLGITIMERSSFEKNPIDFLEAKGYKEVKKDLIIKLPKYSLFELENGRKRMLASAGELQKGNELALPSKYVNFLYLASHYEKLKGSPEDNEQKQLFVEQHKHYLDEIIEQISEFSKRVILADANLDKVLSAYNKHRDKPIREQAENIIHLFTLTNLGAPAAFKYFDTTIDRKRYTSTKEVLDATLIHQSITGLYETRIDLSQLGGD

SEQ ID NO: 7 - protein, 1380 aa, Artificial Sequence
  C80L mutant of dCas9 for dCas9-biotin
MGSSHHHHHHSSGDKKYSIGLAIGTNSVGWAVITDEYKVPSKKFKVLGNTDRHSIKKNLIGALLFDSGETAEATRLKRTARRRYTRRKNRILYLQEIFSNEMAKVDDSFFHRLEESFLVEEDKKHERHPIFGNIVDEVAYHEKYPTIYHLRKKLVDSTDKADLRLIYLALAHMIKFRGHFLIEGDLNPDNSDVDKLFIQLVQTYNQLFEENPINASGVDAKAILSARLSKSRRLENLIAQLPGEKKNGLFGNLIALSLGLTPNFKSNFDLAEDAKLQLSKDTYDDDLDNLLAQIGDQYADLFLAAKNLSDAILLSDILRVNTEITKAPLSASMIKRYDEHHQDLTLLKALVRQQLPEKYKEIFFDQSKNGYAGYIDGGASQEEFYKFIKPILEKMDGTEELLVKLNREDLLRKQRTFDNGSIPHQIHLGELHAILRRQEDFYPFLKDNREKIEKILTFRIPYYVGPLARGNSRFAWMTRKSEETITPWNFEEVVDKGASAQSFIERMTNFDKNLPNEKVLPKHSLLYEYFTVYNELTKVKYVTEGMRKPAFLSGEQKKAIVDLLFKTNRKVTVKQLKEDYFKKIECFDSVEISGVEDRFNASLGTYHDLLKIIKDKDFLDNEENEDILEDIVLTLTLFEDREMIEERLKTYAHLFDDKVMKQLKRRRYTGWGRLSRKLINGIRDKQSGKTILDFLKSDGFANRNFMQLIHDDSLTFKEDIQKAQVSGQGDSLHEHIANLAGSPAIKKGILQTVKVVDELVKVMGRHKPENIVIEMARENQTTQKGQKNSRERMKRIEEGIKELGSQILKEHPVENTQLQNEKLYLYYLQNGRDMYVDQELDINRLSDYDVDAIVPQSFLKDDSIDNKVLTRSDKNRGKSDNVPSEEVVKKMKNYWRQLLNAKLITQRKFDNLTKAERGGLSELDKAGFIKRQLVETRQITKHVAQILDSRMNTKYDENDKLIREVKVITLKSKLVSDFRKDFQFYKVREINNYHHAHDAYLNAVVGTALIKKYPKLESEFVYGDYKVYDVRKMIAKSEQEIGKATAKYFFYSNIMNFFKTEITLANGEIRKRPLIETNGETGEIVWDKGRDFATVRKVLSMPQVNIVKKTEVQTGGFSKESILPKRNSDKLIARKKDWDPKKYGGFDSPTVAYSVLVVAKVEKGKSKKLKSVKELLGITIMERSSFEKNPIDFLEAKGYKEVKKDLIIKLPKYSLFELENGRKRMLASAGELQKGNELALPSKYVNFLYLASHYEKLKGSPEDNEQKQLFVEQHKHYLDEIIEQISEFSKRVILADANLDKVLSAYNKHRDKPIREQAENIIHLFTLTNLGAPAAFKYFDTTIDRKRYTSTKEVLDATLIHQSITGLYETRIDLSQLGGD

SEQ ID NO: 8 - protein, 1380 aa, Artificial Sequence
  C574E mutant of dCas9 for dCas9-biotin
MGSSHHHHHHSSGDKKYSIGLAIGTNSVGWAVITDEYKVPSKKFKVLGNTDRHSIKKNLIGALLFDSGETAEATRLKRTARRRYTRRKNRICYLQEIFSNEMAKVDDSFFHRLEESFLVEEDKKHERHPIFGNIVDEVAYHEKYPTIYHLRKKLVDSTDKADLRLIYLALAHMIKFRGHFLIEGDLNPDNSDVDKLFIQLVQTYNQLFEENPINASGVDAKAILSARLSKSRRLENLIAQLPGEKKNGLFGNLIALSLGLTPNFKSNFDLAEDAKLQLSKDTYDDDLDNLLAQIGDQYADLFLAAKNLSDAILLSDILRVNTEITKAPLSASMIKRYDEHHQDLTLLKALVRQQLPEKYKEIFFDQSKNGYAGYIDGGASQEEFYKFIKPILEKMDGTEELLVKLNREDLLRKQRTFDNGSIPHQIHLGELHAILRRQEDFYPFLKDNREKIEKILTFRIPYYVGPLARGNSRFAWMTRKSEETITPWNFEEVVDKGASAQSFIERMTNFDKNLPNEKVLPKHSLLYEYFTVYNELTKVKYVTEGMRKPAFLSGEQKKAIVDLLFKTNRKVTVKQLKEDYFKKIEEFDSVEISGVEDRFNASLGTYHDLLKIIKDKDFLDNEENEDILEDIVLTLTLFEDREMIEERLKTYAHLFDDKVMKQLKRRRYTGWGRLSRKLINGIRDKQSGKTILDFLKSDGFANRNFMQLIHDDSLTFKEDIQKAQVSGQGDSLHEHIANLAGSPAIKKGILQTVKVVDELVKVMGRHKPENIVIEMARENQTTQKGQKNSRERMKRIEEGIKELGSQILKEHPVENTQLQNEKLYLYYLQNGRDMYVDQELDINRLSDYDVDAIVPQSFLKDDSIDNKVLTRSDKNRGKSDNVPSEEVVKKMKNYWRQLLNAKLITQRKFDNLTKAERGGLSELDKAGFIKRQLVETRQITKHVAQILDSRMNTKYDENDKLIREVKVITLKSKLVSDFRKDFQFYKVREINNYHHAHDAYLNAVVGTALIKKYPKLESEFVYGDYKVYDVRKMIAKSEQEIGKATAKYFFYSNIMNFFKTEITLANGEIRKRPLIETNGETGEIVWDKGRDFATVRKVLSMPQVNIVKKTEVQTGGFSKESILPKRNSDKLIARKKDWDPKKYGGFDSPTVAYSVLVVAKVEKGKSKKLKSVKELLGITIMERSSFEKNPIDFLEAKGYKEVKKDLIIKLPKYSLFELENGRKRMLASAGELQKGNELALPSKYVNFLYLASHYEKLKGSPEDNEQKQLFVEQHKHYLDEIIEQISEFSKRVILADANLDKVLSAYNKHRDKPIREQAENIIHLFTLTNLGAPAAFKYFDTTIDRKRYTSTKEVLDATLIHQSITGLYETRIDLSQLGGD

SEQ ID NO: 9 - DNA, 579 bp, Artificial Sequence
  exogenous human erythropoietin gene
atgggggtgcacgaatgtcctgcctggctgtggcttctcctgtccctgctgtcgctccctctgggcctcccagtcctgggcgccccaccacgcctcatctgtgacagccgagtcctggagaggtacctcttggaggccaaggaggccgagaatatcacgacgggctgtgctgaacactgcagcttgaatgagaatatcactgtcccagacaccaaagttaatttctatgcctggaagaggatggaggtcgggcagcaggccgtagaagtctggcagggcctggccctgctgtcggaagctgtcctgcggggccaggccctgttggtcaactcttcccagccgtgggagcccctgcagctgcatgtggataaagccgtcagtggccttcgcagcctcaccactctgcttcgggctctgggagcccagaaggaagccatctcccctccagatgcggcctcagctgctccactccgaacaatcactgctgacactttccgcaaactcttccgagtctactccaatttcctccggggaaagctgaagctgtacacaggggaggcctgcaggacaggggacaga